European Patent Application EP 4 303 227 A1, published January 10, 2024. Title: Method for preparing proteins with supramolecular structures encapsulating bioactive substances. Applicant: AJINOMOTO CO., INC. The sequence listing filed with the application follows.

SEQUENCE LISTING (4 sequences)

SEQ ID NO: 1 - RNA, 27 nt, Artificial Sequence
  RNA
ggcgcugccaaggcugugggcaagguc

SEQ ID NO: 2 - RNA, 27 nt, Artificial Sequence
  RNA
gaccuugcccacagccuuggcagcguc

SEQ ID NO: 3 - protein, 19 aa, Artificial Sequence
  Peptide
MNVITNLLAGVVHFLGWLV

SEQ ID NO: 4 - protein, 8 aa, Artificial Sequence
  Peptide
GFILGFIL